European Patent Application EP 4 527 854 A2, published March 26, 2025. Title: ANTIBODIES AGAINST PD-L1. Applicant: GENMAB A/S. Application EP. The sequence listing filed with the application follows.

SEQUENCE LISTING (115 sequences)

SEQ ID NO: 1 - protein, 119 aa, synthetic construct
EVQVVESGGGLVQPGGSLRLSCAASGFTFSRFWMSWVRQAPGKGLEWVANIKQDGGEKYYVDSVKGRFTISRDNAKNSLYLQMNSLRGEDTAVYYCARDDNWNGHFDYWGQGTLVTVSS

SEQ ID NO: 2 - protein, 8 aa, synthetic construct
GFTFSRFW

SEQ ID NO: 3 - protein, 8 aa, synthetic construct
IKQDGGEK

SEQ ID NO: 4 - protein, 12 aa, synthetic construct
ARDDNWNGHFDY

SEQ ID NO: 5 - protein, 107 aa, synthetic construct
DIQMTQSPSTLSASVGDRVTITCRASQSISSWLAWYQQKPGKAPNLLIYKASSLESGVPSRFSGSGSGTEFTLTISSLQPDDFATYYCQQYYGSYITFGQGTRLEIK

SEQ ID NO: 6 - protein, 6 aa, synthetic construct
QSISSW

SEQ ID NO: 7 - protein, 9 aa, synthetic construct
QQYYGSYIT

SEQ ID NO: 8 - protein, 121 aa, synthetic construct
QVQLVQSGSELKKPGASVMVSCKASGYTFTSYVMNWVRQAPGQGLEWMGWINSYTGNPTSAQGFTGRFVFSFDTSVNTAYLQISSLKAEDTAVYYCARGYCTSTSCYLDYWGQGTLVTVSS

SEQ ID NO: 9 - protein, 8 aa, synthetic construct
GYTFTSYV

SEQ ID NO: 10 - protein, 8 aa, synthetic construct
INSYTGNP

SEQ ID NO: 11 - protein, 14 aa, synthetic construct
ARGYCTSTSCYLDY

SEQ ID NO: 12 - protein, 108 aa, synthetic construct
SYELTQPPSVSVSPGHTARITCSGDALPKKYACWFQQKSGQAPVLVIYEDSKRPSGIPERFSGSTSGTMATLTISGAQVEDETDYYCYSADTSGTHRVFGGGTKLTVL

SEQ ID NO: 13 - protein, 6 aa, synthetic construct
ALPKKY

SEQ ID NO: 14 - protein, 11 aa, synthetic construct
YSADTSGTHRV

SEQ ID NO: 15 - protein, 108 aa, synthetic construct
  REGION 1..108: note = N/A
SYELTQPPSVSVSPGHTARITCSGDALPKKYASWFQQKSGQAPVLVIYEDSKRPSGIPERFSGSTSGTMATLTISGAQVEDETDYYCYSADTSGTHRVFGGGTKLTVL

SEQ ID NO: 16 - protein, 6 aa, synthetic construct
ALPKKY

SEQ ID NO: 17 - protein, 11 aa, synthetic construct
YSADTSGTHRV

SEQ ID NO: 18 - protein, 121 aa, synthetic construct
EVQLLEPGGGLVQPGGSLRLSCEASGSTFSTYAMSWVRQAPGKGLEWVSGFSGSGGFTFYADSVRGRFTISRDSSKNTLFLQMSSLRAEDTAVYYCAIPARGYNYGSFQHWGQGTLVTVSS

SEQ ID NO: 19 - protein, 8 aa, synthetic construct
GSTFSTYA

SEQ ID NO: 20 - protein, 8 aa, synthetic construct
FSGSGGFT

SEQ ID NO: 21 - protein, 14 aa, synthetic construct
AIPARGYNYGSFQH

SEQ ID NO: 22 - protein, 108 aa, synthetic construct
SYVLTQPPSVSVAPGQTARITCGGNNIGSKSVHWYQQKPGQAPVLVVYDDNDRPSGLPERFSGSNSGNTATLTISRVEAGDEADYYCQVWDSSSDHVVFGGGTKLTVL

SEQ ID NO: 23 - protein, 6 aa, synthetic construct
NIGSKS

SEQ ID NO: 24 - protein, 11 aa, synthetic construct
QVWDSSSDHVV

SEQ ID NO: 25 - protein, 125 aa, synthetic construct
EVKLVESGGGLVQPGGSLRLSCAASGFTFNTYAMNWVRQAPGKGLEWVARIRSKYNNYATYYADSVKDRFTISRDDSKSSLYLQMNNLKTEDTAMYYCVRHGNFGNSYVSWFAYWGQGTLVTVSS

SEQ ID NO: 26 - protein, 8 aa, synthetic construct
GFTFNTYA

SEQ ID NO: 27 - protein, 10 aa, synthetic construct
IRSKYNNYAT

SEQ ID NO: 28 - protein, 16 aa, synthetic construct
VRHGNFGNSYVSWFAY

SEQ ID NO: 29 - protein, 109 aa, synthetic construct
QAVVTQEPSFSVSPGGTVTLTCRSSTGAVTTSNYANWVQQTPGQAFRGLIGGTNKRAPGVPARFSGSLIGDKAALTITGAQADDESIYFCALWYSNLWVFGGGTKLTVL

SEQ ID NO: 30 - protein, 9 aa, synthetic construct
TGAVTTSNY

SEQ ID NO: 31 - protein, 9 aa, synthetic construct
ALWYSNLWV

SEQ ID NO: 32 - protein, 123 aa, synthetic construct
EVQLVESGGGLVQPGGSLRLSCAASGFTFSSYWMSWVRQAPGKGLEWVANIKQDGNEKYYVDSVKGRFTISRDNAKNSLYVQMNSLRAEDTAVYYCARDLYYGSGTYPPFDYWGQGTLVTVSS

SEQ ID NO: 33 - protein, 8 aa, synthetic construct
GFTFSSYW

SEQ ID NO: 34 - protein, 8 aa, synthetic construct
IKQDGNEK

SEQ ID NO: 35 - protein, 16 aa, synthetic construct
ARDLYYGSGTYPPFDY

SEQ ID NO: 36 - protein, 107 aa, synthetic construct
DIQMTQSPSTLSASVGDRVTITCRASQSISSWLAWYLQKPGKAPKLLIYKASSLESGVPSRFSGSGSGTEFTLTISSLQPDDFATYYCQQYHSSSYTFGQGTKLEIK

SEQ ID NO: 37 - protein, 6 aa, synthetic construct
QSISSW

SEQ ID NO: 38 - protein, 9 aa, synthetic construct
QQYHSSSYT

SEQ ID NO: 39 - protein, 125 aa, synthetic construct
  REGION 1..125: note = N/A
EVKLVESGGGLVQPGGSLRLSCAASGFTFNPYAMNWVRQAPGKGLEWVARIRSKYNNYATYYADSVKDRFTISRDDSKSSLYLQMNNLKTEDTAMYYCVRHGNFGNSYVSWFAYWGQGTLVTVSS

SEQ ID NO: 40 - protein, 125 aa, synthetic construct
EVKLVESGGGLVQPGGSLRLSCAASGFTFNMYAMNWVRQAPGKGLEWVARIRSKYNNYATYYADSVKDRFTISRDDSKSSLYLQMNNLKTEDTAMYYCVRHGNFGNSYVSWFAYWGQGTLVTVSS

SEQ ID NO: 41 - protein, 126 aa, synthetic construct
  REGION 1..126: note = N/A
EVKLVESGGGLVQPGGSLRLSCAASGFTFNTYAMNWVRQAPGKGLEWVARIRSKYNNYATYYADSVKDRFTISRDDSKSSLYLQMNNLKTEDTAMYYCVRHGNFGNSYVSWFAYVWGQGTLVTVSS

SEQ ID NO: 42 - protein, 125 aa, synthetic construct
  REGION 1..125: note = N/A
EVKLVESGGGLVQPGGSLRLSCAASGFTFNTYAMNWVRQAPGKGLEWVARIRSKYNNYATYYADSVKDRFTISRDDSKSSLYLQMNNLKTEDTAMYYCVRHGNFGNSYVSWFAMWGQGTLVTVSS

SEQ ID NO: 43 - protein, 125 aa, synthetic construct
  REGION 1..125: note = N/A
EVKLVESGGGLVQPGGSLRLSCAASGFTFNTYAMNWVRQAPGKGLEWVARIRSKYNNYATYYADSVKDRFTISRDDSKSSLYLQMNNLKTEDTAMYYCVRHGNFGNSYVSWFARWGQGTLVTVSS

SEQ ID NO: 44 - protein, 125 aa, synthetic construct
  REGION 1..125: note = N/A
EVKLVESGGGLVQPGGSLRLSCAASGFTFNTYAMNWVRQAPGKGLEWVARIRSKYNNYATYYADSVKDRFTISRDDSKSSLYLQMNNLKTEDTAMYYCVRHGNFGNSYVAWFAYWGQGTLVTVSS

SEQ ID NO: 45 - protein, 125 aa, synthetic construct
  REGION 1..125: note = N/A
EVKLVESGGGLVQPGGSLRLSCAASGFTFNTYAMNWVRQAPGKGLEWVARIRSKYNNYATYYADSVKDRFTISRDDSKSSLYLQMNNLKTEDTAMYYCVRGGNFGNSYVSWFAYWGQGTLVTVSS

SEQ ID NO: 46 - protein, 121 aa, synthetic construct
EVQLVESGGGLVQPGRSLRLSCAASGFTFDDYAMHWVRQGPGKGLEWVSGIRWNSGSMHYADSVKGRFTISRDNAKSSLYLQMNSLRAEDTALYYCARAPWYSGAWHPDYWGQGTLVTVSS

SEQ ID NO: 47 - protein, 8 aa, synthetic construct
GFTFDDYA

SEQ ID NO: 48 - protein, 8 aa, synthetic construct
IRWNSGSM

SEQ ID NO: 49 - protein, 14 aa, synthetic construct
ARAPWYSGAWHPDY

SEQ ID NO: 50 - protein, 110 aa, synthetic construct
  REGION 1..110: note = N/A
QSALTQPRSVSGSPGQSVTISCTGTSSDVGTYNYVSWYQQHPGKAPKLMIYDVIKRPSGVPDRFSGSKSGNTASLTLSGLQAEDEADYYCSSYAGTYTLLFGGGTKLTVL

SEQ ID NO: 51 - protein, 9 aa, synthetic construct
SSDVGTYNY

SEQ ID NO: 52 - protein, 10 aa, synthetic construct
  REGION 1..10: note = N/A
SSYAGTYTLL

SEQ ID NO: 53 - protein, 127 aa, synthetic construct
  REGION 1..127: note = N/A
EVQMLESGGGLVQPGGSLRLSCAASGFTFRSYAMSWVRQAPGKGLEWVSGIGDSGGSTYHADSVKGRFTISRDNSKNTLYLQMNSLRAEDTAVYYCAKLGQSSGWYDHYYYYGMDVWGQGTTVTVSS

SEQ ID NO: 54 - protein, 8 aa, synthetic construct
GFTFRSYA

SEQ ID NO: 55 - protein, 8 aa, synthetic construct
IGDSGGST

SEQ ID NO: 56 - protein, 20 aa, synthetic construct
  REGION 1..20: note = N/A
AKLGQSSGWYDHYYYYGMDV

SEQ ID NO: 57 - protein, 106 aa, synthetic construct
  REGION 1..106: note = N/A
SYELTQPPSVSVSPGQTASITCSGDKLGNKYVSWFQQKPGQSPVLVIYRDSERPSGIPERFSGSNSGNTATLTISGTQAVDEADFYCQAWDSSTVVFGGGTKLTVL

SEQ ID NO: 58 - protein, 6 aa, synthetic construct
KLGNKY

SEQ ID NO: 59 - protein, 9 aa, synthetic construct
QAWDSSTVV

SEQ ID NO: 60 - protein, 120 aa, synthetic construct
QVQLQESGPGLVKPSDTLSLTCAVSDYSISSNDWWGWIRQPPGKGLEWIGYIYYSGTGYYNPSLKSRVTISIDTSKNQFSLKLNSVTAVDTAVYYCARTRVGARRAFDYWGQGTLVTVSS

SEQ ID NO: 61 - protein, 9 aa, synthetic construct
DYSISSNDW

SEQ ID NO: 62 - protein, 7 aa, synthetic construct
IYYSGTG

SEQ ID NO: 63 - protein, 13 aa, synthetic construct
ARTRVGARRAFDY

SEQ ID NO: 64 - protein, 108 aa, synthetic construct
SYVLTQPPSVSVAPGQTARITCGGNNIGSKSVHWYQQKPGQAPVLVVYDDSDRPSGIPERFSGSNSGNTATLTISRVEAGDEADYYCQVWDSSSDHVVFGGGTKLTVL

SEQ ID NO: 65 - protein, 6 aa, synthetic construct
NIGSKS

SEQ ID NO: 66 - protein, 11 aa, synthetic construct
QVWDSSSDHVV

SEQ ID NO: 67 - protein, 123 aa, synthetic construct
QVQLVESGGGLVKPGGSLRLSCAASGFTFSDYYMSWIRQAPGKGLEWVSYIGSSSNTIYYADSVKGRFTISRDNAKNSLYLQMNSLRAEDTAVYSCARDRVKYGSPGSLFDYWGQGTLVTVSS

SEQ ID NO: 68 - protein, 8 aa, synthetic construct
GFTFSDYY

SEQ ID NO: 69 - protein, 8 aa, synthetic construct
IGSSSNTI

SEQ ID NO: 70 - protein, 16 aa, synthetic construct
ARDRVKYGSPGSLFDY

SEQ ID NO: 71 - protein, 108 aa, synthetic construct
SYELTQPPSVSVSPGQTARITCSGDALPKKYAFWYQQKSGQAPVLVIYEDSKRPSGIPERFSGSSSGTMATLTISGAQVEDEADYYCYSTASSGDHRVFGGGTKLTVL

SEQ ID NO: 72 - protein, 6 aa, synthetic construct
ALPKKY

SEQ ID NO: 73 - protein, 11 aa, synthetic construct
YSTASSGDHRV

SEQ ID NO: 74 - protein, 118 aa, synthetic construct
EVQLVESGGGLVQPGGSLRLSCAASGFTFSDSWIHWYRQAPGKGLEWYAWISPYGGSTYYADSVKGRFTISADTSKNTAYLQMNSLRAEDTAVYYCARRHWPGGFDYWGQGTLVTVSS

SEQ ID NO: 75 - protein, 8 aa, synthetic construct
GFTFSDSW

SEQ ID NO: 76 - protein, 8 aa, synthetic construct
ISPYGGST

SEQ ID NO: 77 - protein, 11 aa, synthetic construct
ARRHWPGGFDY

SEQ ID NO: 78 - protein, 107 aa, synthetic construct [sequence omitted]

SEQ ID NO: 79 - protein, 6 aa, synthetic construct
QDVSTA

SEQ ID NO: 80 - protein, 9 aa, synthetic construct
QQYLYHPAT

SEQ ID NO: 81 - protein, 121 aa, synthetic construct
EVQLVESGGGLVQPGGSLRLSCAASGFTFSRYWMSWVRQAPGKGLEWVANIKQDGSEKYYVDSVKGRFTISRDNAKNSLYLQMNSLRAEDTAVYYCAREGGWFGELAFDYWGQGTLVTVSS

SEQ ID NO: 82 - protein, 8 aa, synthetic construct
GFTFSRYW

SEQ ID NO: 83 - protein, 8 aa, synthetic construct
IKQDGSEK

SEQ ID NO: 84 - protein, 14 aa, synthetic construct
AREGGWFGELAFDY

SEQ ID NO: 85 - protein, 108 aa, synthetic construct
EIVLTQSPGTLSLSPGERATLSCRASQRVSSSYLAWYQQKPGQAPRLLIYDASSRATGIPDRFSGSGSGTDFTLTISRLEPEDFAVYYCQQYGSLPWTFGQGTKVEIK

SEQ ID NO: 86 - protein, 7 aa, synthetic construct
QRVSSSY

SEQ ID NO: 87 - skipped

SEQ ID NO: 88 - protein, 9 aa, synthetic construct
QQYGSLPWT

SEQ ID NO: 89 - protein, 330 aa, synthetic construct
  REGION 1..330: note = N/A
ASTKGPSVFPLAPSSKSTSGGTAALGCLVKDYFPEPVTVSWNSGALTSGVHTFPAVLQSSGLYSLSSVVTVPSSSLGTQTYICNVNHKPSNTKVDKRVEPKSCDKTHTCPPCPAPEFEGGPSVFLFPPKPKDTLMISRTPEVTCVVVAVSHEDPEVKFNWYVDGVEVHNAKTKPREEQYNSTYRVVSVLTVLHQDWLNGKEYKCKVSNKALPAPIEKTISKAKGQPREPQVYTLPPSREEMTKNQVSLTCLVKGFYPSDIAVEWESNGQPENNYKTTPPVLDSDGSFFLYSRLTVDKSRWQQGNVFSCSVMHEALHNHYTQKSLSLSPGK

SEQ ID NO: 90 - protein, 330 aa, synthetic construct
  REGION 1..330: note = N/A
ASTKGPSVFPLAPSSKSTSGGTAALGCLVKDYFPEPVTVSWNSGALTSGVHTFPAVLQSSGLYSLSSVVTVPSSSLGTQTYICNVNHKPSNTKVDKRVEPKSCDKTHTCPPCPAPEFEGGPSVFLFPPKPKDTLMISRTPEVTCVVVAVSHEDPEVKFNWYVDGVEVHNAKTKPREEQYNSTYRVVSVLTVLHQDWLNGKEYKCKVSNKALPAPIEKTISKAKGQPREPQVYTLPPSREEMTKNQVSLTCLVKGFYPSDIAVEWESNGQPENNYKTTPPVLDSDGSFLLYSKLTVDKSRWQQGNVFSCSVMHEALHNHYTQKSLSLSPGK

SEQ ID NO: 91 - protein, 107 aa, Homo sapiens [sequence omitted]

SEQ ID NO: 92 - protein, 106 aa, Homo sapiens
GQPKAAPSVTLFPPSSEELQANKATLVCLISDFYPGAVTVAWKADSSPVKAGVETTTPSKQSNNKYAASSYLSLTPEQWKSHRSYSCQVTHEGSTVEKTVAPTECS

SEQ ID NO: 93 - protein, 330 aa, Homo sapiens
ASTKGPSVFPLAPSSKSTSGGTAALGCLVKDYFPEPVTVSWNSGALTSGVHTFPAVLQSSGLYSLSSVVTVPSSSLGTQTYICNVNHKPSNTKVDKRVEPKSCDKTHTCPPCPAPELLGGPSVFLFPPKPKDTLMISRTPEVTCVVVDVSHEDPEVKFNWYVDGVEVHNAKTKPREEQYNSTYRVVSVLTVLHQDWLNGKEYKCKVSNKALPAPIEKTISKAKGQPREPQVYTLPPSREEMTKNQVSLTCLVKGFYPSDIAVEWESNGQPENNYKTTPPVLDSDGSFFLYSKLTVDKSRWQQGNVFSCSVMHEALHNHYTQKSLSLSPGK

SEQ ID NO: 94 - protein, 290 aa, Homo sapiens
MRIFAVFIFMTYWHLLNAFTVTVPKDLYVVEYGSNMTIECKFPVEKQLDLAALIVYWEMEDKNIIQFVHGEEDLKVQHSSYRQRARLLKDQLSLGNAALQITDVKLQDAGVYRCMISYGGADYKRITVKVNAPYNKINQRILVVDPVTSEHELTCQAEGYPKAEVIWTSSDHQVLSGKTTTTNSKREEKLFNVTSTLRINTTTNEIFYCTFRRLDPEENHTAELVIPELPLAHPPNERTHLVILGAILLCLGVALTFIFRLRKGRMMDVKKCGIQDTNSKKQSDTHLEET

SEQ ID NO: 95 - protein, 186 aa, Homo sapiens
QDGNEEMGGITQTPYKVSISGTTVILTCPQYPGSEILWQHNDKNIGGDEDDKNIGSDEDHLSLKEFSELEQSGYYVCYPRGSKPEDANFYLYLRARVCENCMEMDVMSVATIVIVDICITGGLLLLVYYWSKNRKAKAKPVTRGAGAGGRQRGQNKERPPPVPNPDYEPIRKGQRDLYSGLNQRRI

SEQ ID NO: 96 - protein, 107 aa, Homo sapiens
GQPREPQVYTLPPSRDELTKNQVSLTCLVKGFYPSDIAVEWESNGQPENNYKTTPPVLDSDGSFFLYSKLTVDKSRWQQGNVFSCSVMHEALHNHYTQKSLSLSPGK

SEQ ID NO: 97 - protein, 107 aa, Homo sapiens
GQPREPQVYTLPPSREEMTKNQVSLTCLVKGFYPSDIAVEWESNGQPENNYKTTPPVLDSDGSFFLYSKLTVDKSRWQQGNVFSCSVMHEALHNHYTQKSLSLSPGK

SEQ ID NO: 98 - protein, 107 aa, Homo sapiens
GQPREPQVYTLPPSRDELTKNQVSLTCLVKGFYPSDIAVEWESNGQPENNYKTTPPVLDSDGSFFLYSKLTVDKSRWQQGNVFSCSVMHEGLHNHYTQKSLSLSPGK

SEQ ID NO: 99 - protein, 8 aa, synthetic construct
  REGION 1..8: note = N/A
GFTFNPYA

SEQ ID NO: 100 - protein, 8 aa, synthetic construct
  REGION 1..8: note = N/A
GFTFNMYA

SEQ ID NO: 101 - protein, 16 aa, synthetic construct
  REGION 1..16: note = N/A
VRHGNFGNSYVSWFAV

SEQ ID NO: 102 - protein, 16 aa, synthetic construct
  REGION 1..16: note = N/A
VRHGNFGNSYVSWFAM

SEQ ID NO: 103 - protein, 16 aa, synthetic construct
  REGION 1..16: note = N/A
VRHGNFGNSYVSWFAR

SEQ ID NO: 104 - protein, 16 aa, synthetic construct
  REGION 1..16: note = N/A
VRHGNFGNSYVAWFAY

SEQ ID NO: 105 - protein, 16 aa, synthetic construct
  REGION 1..16: note = N/A
VRGGNFGNSYVSWFAY

SEQ ID NO: 106 - protein, 124 aa, synthetic construct
HMQLVESGGGVAQPGRSLRLSCAASGFTFSNYGMHWVRQAPGRGLEWLAVMSYDGETKYYADSVKGRFTISRDNSENTLFLQMNSLRAEDTAVYYCAKDTSNGWNYYFYGMDVWGQGTTVTVSS

SEQ ID NO: 107 - protein, 8 aa, synthetic construct
GFTFSNYG

SEQ ID NO: 108 - protein, 8 aa, synthetic construct
MSYDGETK

SEQ ID NO: 109 - protein, 17 aa, synthetic construct
AKDTSNGWNYYFYGMDV

SEQ ID NO: 110 - protein, 108 aa, synthetic construct
SYELTQPPSVSVSPGQTARITCSGDALPKKFASWYQQKSGQAPVLVIYEDSKRPSGIPERVSGSSSGTMATLTISGAQTEDEADYYCYSTDRSGYHWVFGGGTKLTVL

SEQ ID NO: 111 - protein, 6 aa, synthetic construct
ALPKKF

SEQ ID NO: 112 - protein, 11 aa, synthetic construct
YSTDRSGYHWV

SEQ ID NO: 113 - protein, 330 aa, Homo sapiens; identical to SEQ ID NO: 93

SEQ ID NO: 114 - protein, 330 aa, synthetic construct
  REGION 1..330: note = N/A
ASTKGPSVFPLAPSSKSTSGGTAALGCLVKDYFPEPVTVSWNSGALTSGVHTFPAVLQSSGLYSLSSVVTVPSSSLGTQTYICNVNHKPSNTKVDKRVEPKSCDKTHTCPPCPAPELLGGPSVFLFPPKPKDTLMISRTPEVTCVVVDVSHEDPEVKFNWYVDGVEVHNAKTKPREEQYNSTYRVVSVLTVLHQDWLNGKEYKCKVSNKALPAPIEKTISKAKGQPREPQVYTLPPSREEMTKNQVSLTCLVKGFYPSDIAVEWESNGQPENNYKTTPPVLDSDGSFFLYSRLTVDKSRWQQGNVFSCSVMHEALHNHYTQKSLSLSPGK

SEQ ID NO: 115 - protein, 330 aa, synthetic construct
  REGION 1..330: note = N/A
ASTKGPSVFPLAPSSKSTSGGTAALGCLVKDYFPEPVTVSWNSGALTSGVHTFPAVLQSSGLYSLSSVVTVPSSSLGTQTYICNVNHKPSNTKVDKRVEPKSCDKTHTCPPCPAPELLGGPSVFLFPPKPKDTLMISRTPEVTCVVVDVSHEDPEVKFNWYVDGVEVHNAKTKPREEQYNSTYRVVSVLTVLHQDWLNGKEYKCKVSNKALPAPIEKTISKAKGQPREPQVYTLPPSREEMTKNQVSLTCLVKGFYPSDIAVEWESNGQPENNYKTTPPVLDSDGSFLLYSKLTVDKSRWQQGNVFSCSVMHEALHNHYTQKSLSLSPGK